European Patent Application EP 4 553 161 A1, published May 14, 2025. Title: 一种无抗性质粒骨架及其生产系统. Applicant: 云舟生物科技（广州）有限公司. The sequence listing filed with the application follows.

SEQUENCE LISTING (19 sequences)

SEQ ID NO: 1 - DNA, 558 bp, synthetic construct
  source 1..558: mol_type = other DNA
gtttaaggaattttgtggctggccacgccgtaaggtggcaaggaactggttctgatgtggatttacaggagccagaaaagcaaaaaccccgataatcttcttcaactttggcgagtacgaaaagattaccggggcccacttaaaccgtatagccaacaattcagctatgcggggagtatagttatatgcccggaaaagttcaagacttctttctgtgctcgctccttctgcgcattgtaagtgcaggatggtgtgcagtttaaggtttacacctataaaagagagagccgttatcgtctgtttgtggatgtacagagtgatattattgacacgcccgggcgacggatggtgatccccctggccagtgcacgtctgctgtcagataaagtctcccgtgaactttacccggtggtgcatatcggggatgaaagctggcgcatgatgaccaccgatatggccagtgtgccggtctccgttatcggggaagaagtggctgatctcagccaccgcgaaaatgacatcaaaaacgccattaacctgatgttctggggaatataa

SEQ ID NO: 2 - DNA, 370 bp, synthetic construct
  source 1..370: mol_type = other DNA
ggtagacacacatcttgtcatatgatataatggtttcgccaaaaatcaataatcagacaacaaggtgcagtttaaggtttacacctataaaagagagagccgttatcgtctgtttgtggatgtacagagtgatattattgacacgcccgggcgacggatggtgatccccctggccagtgcacgtctgctgtcagataaagtctcccgtgaactttacccggtggtgcatatcggggatgaaagctggcgcatgatgaccaccgatatggccagtgtgccggtctccgttatcggggaagaagtggctgatctcagccaccgcgaaaatgacatcaaaaacgccattaacctgatgttctggggaatataa

SEQ ID NO: 3 - DNA, 258 bp, synthetic construct
  source 1..258: mol_type = other DNA
agtcacaccatcctgcacttacaatgcgcagaaggagcgagcacagaaagaagtcttgaacttttccgggcatataactatactccccgcatagctgaattgttggctatacggtttaagtgggccccggtaatcttttcgtactcgccaaagttgaagaagattatcggggtttttgcttttctggctcctgtaaatccacatcagaaccagttccttgccaccttacggcgtggccagccacaaaattccttaaac

SEQ ID NO: 4 - DNA, 229 bp, synthetic construct
  source 1..229: mol_type = other DNA
agaaggagcgagcacagaaagaagtcttgaacttttccgggcatataactatactccccgcatagctgaattgttggctatacggtttaagtgggccccggtaatcttttcgtactcgccaaagttgaagaagattatcggggtttttgcttttctggctcctgtaaatccacatcagaaccagttccttgccaccttacggcgtggccagccacaaaattccttaaac

SEQ ID NO: 5 - DNA, 181 bp, synthetic construct
  source 1..181: mol_type = other DNA
agaaggagcgagcacagaaagaagtcttgaacttttccgggcatataactatactccccgcatagctgaattgttggctatacggtttaagtgggccccggtaatcttttcgtactcgccaaagttgaagaagattatcggggtttttgcttttctggctcctgtaaatccacatcagaac

SEQ ID NO: 6 - DNA, 154 bp, synthetic construct
  source 1..154: mol_type = other DNA
agaaggagcgagcacagaaagaagtcttgaacttttccgggcatataactatactccccgcatagctgaattgttggctatacggtttaagtgggccccggtaatcttttcgtactcgccaaagttgaagaagattatcggggtttttgctttt

SEQ ID NO: 7 - DNA, 123 bp, synthetic construct
  source 1..123: mol_type = other DNA
cttttccgggcatataactatactccccgcatagctgaattgttggctatacggtttaagtgggccccggtaatcttttcgtactcgccaaagttgaagaagattatcggggtttttgctttt

SEQ ID NO: 8 - DNA, 139 bp, synthetic construct
  source 1..139: mol_type = other DNA
gtagaattggtaaagagagtcgtgtaaaatatcgagttcgcacatcttgttgtctgattattgatttttggcgaaaccatttgatcatatgacaagatgtgtatctaccttaacttaatgattttgataaaaatcatta

SEQ ID NO: 9 - DNA, 1813 bp, synthetic construct
  source 1..1813: mol_type = other DNA
gcccgtcacgggcttctcagggcgttttatggcgggtctgctatgtggtgttatctgactttttgctgttcagcagttcctgccctctgattttccagtctgaccacttcggattatcccgtgacaggtcattcagactggctaatgcacccagtaaggcagcggtatcatcaacaggcttacccgtcttactgtctagactcgaggaattgatatcacccgacaccatcgaatggtcaccagtccctgttctcgtcagcaaaagagccgttcatttcaataaaccgggcgacctcagccatcccttcctgattttccgctttccagcgttcggcacgcagacgacgggcttcattctgcatggttgtgcttaccagaccggagatattgacatcatatgccttgagcaactgatagctgtcgctgtcaactgtcactgtaatacgctgcttcatagtgaattcctcctgctagcccaaaaaaacgggtatggagaaacagtagagagttgcgataaaaagcgtcaggtaggatccgctaatcttatggataaaaatgctatggcatagcaaagtgtgacgccgtgcaaataatcaatgtggacttttctgccgtgattatagacacttttgttacgcgtttttgtcatggctttggtcccgctttgttacagaatgcttttaataagcggggttaccggtttggttagcgagaagagccagtaaaagacgcagtgacggcaatgtctgatgcaatatggacaattggtttcttctctgaatggcgggagtatgaaaagtatggctgaagcgcaaaatgatcccctgctgccgggatactcgtttaatgcccatctggtggcgggtttaacgccgattgaggccaacggttatctcgatttttttatcgaccgaccgctgggaatgaaaggttatattctcaatctcaccattcgcggtcagggggtggtgaaaaatcagggacgagaatttgtttgccgaccgggtgatattttgctgttcccgccaggagagattcatcactacggtcgtcatccggaggctcgcgaatggtatcaccagtgggtttactttcgtccgcgcgcctactggcatgaatggcttaactggccgtcaatatttgccaatacggggttctttcgcccggatgaagcgcaccagccgcatttcagcgacctgtttgggcaaatcattaacgccgggcaaggggaagggcgctattcggagctgctggcgataaatctgcttgagcaattgttactgcggcgcatggaagcgattaacgagtcgctccatccaccgatggataatcgggtacgcgaggcttgtcagtacatcagcgatcacctggcagacagcaattttgatatcgccagcgtcgcacagcatgtttgcttgtcgccgtcgcgtctgtcacatcttttccgccagcagttagggattagcgtcttaagctggcgcgaggaccaacgtatcagccaggcgaagctgcttttgagcaccacccggatgcctatcgccaccgtcggtcgcaatgttggttttgacgatcaactctatttctcgcgggtatttaaaaaatgcaccggggccagcccgagcgagttccgtgccggttgtgaagaaaaagtgaatgatgtagccgtcaagttgtcataattggtaacgaatcagacaattgacggcttgacggagtagcatagggtttgcagaatccctgcttcgtccatttgacaggcacattatgcatcttggagtggtgaatccgttagcgaggtgccgccggcttccat

SEQ ID NO: 10 - DNA, 130 bp, synthetic construct
  source 1..130: mol_type = other DNA
aaaaacaaacgccccgtaaatcgtgctctcaccgccaagattgatcacgaaattacagggcgccgggttccgcgtttcccgatgggaaagcgcggttagttaaactgtgtaccgagagaaatcgtatcac

SEQ ID NO: 11 - DNA, 228 bp, synthetic construct
  source 1..228: mol_type = other DNA
ccgtacgcgaaatcgttcgtacagtacggtttgtgcggtaatttttccctgaagcgttgaagtacggcgctcatgtgatacgatttctctcggtacacagtttaactaaccgcgctttcccatcgggaaacgcggaacccggcgccctgtaatttcgtgatcaatcttggcggtgagagcacgatttacggggcgtttgtttttcagtcgcttacactacacccaacg

SEQ ID NO: 12 - DNA, 262 bp, synthetic construct
  source 1..262: mol_type = other DNA
agataatacaaatgcttaaataaaaaaagacttgatctgattagaccaaatcttttgatagtgttatattaataacaaaataaaaaggagtcgctcacgccctgaccaaagtttgtgaacgacatcattcaaagaaaaaaacactgagttgtttttataatcttgtatatttagatattaaacgatatttaaatatacatcaagatatatatttgggtgagcgattccttaaacgaaattgagattaaggagtcgatttttt

SEQ ID NO: 13 - DNA, 280 bp, synthetic construct
  source 1..280: mol_type = other DNA
cgactccttaatctcaatttcgtttaaggaatcgctcacccaaatatatatcttgatgtatatttaaatatcgtttaatatctaaatatacaagattataaaaacaactcagtgtttttttctttgaatgatgtcgttcacaaactttggtcagggcgtgagcgactcctttttattttgttattaatataacactatcaaaagatttggtctaatcagatcaagtctttttttatttaagcatttgtattatctggtaaacagttaaaactactaaaac

SEQ ID NO: 14 - DNA, 176 bp, synthetic construct
  source 1..176: mol_type = other DNA
cccggcgcttgaggctttctgcctcatgacgtgaaggtggtttgttgccgtgttgtgtggcagaaagaagatagccccgtagtaagttaattttcattaaccaccacgaggcatccctatgtctagtccacatcaggatagcctcttaccgcgctttgcgcaaggagaagaaggcc

SEQ ID NO: 15 - DNA, 342 bp, synthetic construct
  source 1..342: mol_type = other DNA
caacacacaccagacaagggaacttcgtggtagtttcatggccttcttctccttgcgcaaagcgcggtaagaggctatcctgatgtggactagacatagggatgcctcgtggtggttaatgaaaattaacttactacggggctatcttctttctgccacacaacacggcaacaaaccaccttcacgtcatgaggcagaaagcctcaagcgccgggcacatcatagcccatatacctgcacgctgaccacactcactttccctgaaaataatccgctcattcagaccgttcacgggaaatccgtgtgattgttgccgcatcacgctgcctcccggagtttgtt

SEQ ID NO: 16 - DNA, 1122 bp, synthetic construct
  source 1..1122: mol_type = other DNA
gtttaaggaattttgtggctggccacgccgtaaggtggcaaggaactggttctgatgtggatttacaggagccagaaaagcaaaaaccccgataatcttcttcaactttggcgagtacgaaaagattaccggggcccacttaaaccgtatagccaacaattcagctatgcggggagtatagttatatgcccggaaaagttcaagacttctttctgtgctcgctccttctgcgcattgtaagtgcaggatggtgtgactgatgcaaatatagtcaattttactgacaaacaatttgagaatcgcttaaatgataatttagaagaattgattcaaggaaaaaaagcggttgaatcgccaaccgcttttttacttggtgggcaaccagggtcagggaaaaccagtttgcgatcagcaatttttgaagaaacacaagggaatgttattgtcattgataatgatacctttaaacaacagcaccctaattttgatgaactagtgaaactttatgaaaaagacgtagtaaaacacgttaccccttattctaatcgcatgacagaagcgatcataagccgtttgagcgatcaagggtataatttggtgatcgaaggtacaggacgaacaacagacgttcctattcaaaccgcaacaatgcttcaagccaaaggttatgaaacaaaaatgtatgtcatggcagtacctaaaatcaactcatatttaggaacaattgaacgatatgaaaccatgtattcagatgatccaatgacagccagggcaacaccaaaacaagcgcatgatattgttgtcaaaaacttaccgaccaatttagaaacccttcataaaacgggcttatttagcgatataaggctatataacagagaaggagtaaaactctattcaagtttggaaacaccttctattagtccaaaagaaaccttagaaaaagaattgaatcgtaaagtatcagggaaagaaattcaaccgactttagaacgaatagagcaaaaaatggttctaaataaacaccaagagacacctgaatttaaagcaattcaacaaaaattggaaagcttgcagccacctacaccaccaatacccaaaacacctaaacttccaggtatttaa

SEQ ID NO: 17 - DNA, 1867 bp, synthetic construct
  source 1..1867: mol_type = other DNA
gcccgtcacgggcttctcagggcgttttatggcgggtctgctatgtggtgttatctgactttttgctgttcagcagttcctgccctctgattttccagtctgaccacttcggattatcccgtgacaggtcattcagactggctaatgcacccagtaaggcagcggtatcatcaacaggcttacccgtcttactgtctagactcgaggaattgatatcacccgacaccatcgaatggttaagccactttctctttattcaaaacttgttttgagtaacgattcattgaccgccaatactcatgaacggcttgtaattcttctaaagaataatcaaaaagatttacacgttttgcaagctttaattggtttaataaattgacttccaataattgagagtcatttttatttaattcatggttcaaaacatagtttaatactcgattataaacgcttgccgataattcgttaatgatctctatttcaaatgttttttcatacgtaactgccatagtgaattcctcctgctagcccaaaaaaacgggtatggagaaacagtagagagttgcgataaaaagcgtcaggtaggatccgctaatcttatggataaaaatgctatggcatagcaaagtgtgacgccgtgcaaataatcaatgtggacttttctgccgtgattatagacacttttgttacgcgtttttgtcatggctttggtcccgctttgttacagaatgcttttaataagcggggttaccggtttggttagcgagaagagccagtaaaagacgcagtgacggcaatgtctgatgcaatatggacaattggtttcttctctgaatggcgggagtatgaaaagtatggctgaagcgcaaaatgatcccctgctgccgggatactcgtttaatgcccatctggtggcgggtttaacgccgattgaggccaacggttatctcgatttttttatcgaccgaccgctgggaatgaaaggttatattctcaatctcaccattcgcggtcagggggtggtgaaaaatcagggacgagaatttgtttgccgaccgggtgatattttgctgttcccgccaggagagattcatcactacggtcgtcatccggaggctcgcgaatggtatcaccagtgggtttactttcgtccgcgcgcctactggcatgaatggcttaactggccgtcaatatttgccaatacggggttctttcgcccggatgaagcgcaccagccgcatttcagcgacctgtttgggcaaatcattaacgccgggcaaggggaagggcgctattcggagctgctggcgataaatctgcttgagcaattgttactgcggcgcatggaagcgattaacgagtcgctccatccaccgatggataatcgggtacgcgaggcttgtcagtacatcagcgatcacctggcagacagcaattttgatatcgccagcgtcgcacagcatgtttgcttgtcgccgtcgcgtctgtcacatcttttccgccagcagttagggattagcgtcttaagctggcgcgaggaccaacgtatcagccaggcgaagctgcttttgagcaccacccggatgcctatcgccaccgtcggtcgcaatgttggttttgacgatcaactctatttctcgcgggtatttaaaaaatgcaccggggccagcccgagcgagttccgtgccggttgtgaagaaaaagtgaatgatgtagccgtcaagttgtcataattggtaacgaatcagacaattgacggcttgacggagtagcatagggtttgcagaatccctgcttcgtccatttgacaggcacattatgcatcttggagtggtgaatccgttagcgaggtgccgccggcttccat

SEQ ID NO: 18 - DNA, 639 bp, synthetic construct
  source 1..639: mol_type = other DNA
gtttaaggaattttgtggctggccacgccgtaaggtggcaaggaactggttctgatgtggatttacaggagccagaaaagcaaaaaccccgataatcttcttcaactttggcgagtacgaaaagattaccggggcccacttaaaccgtatagccaacaattcagctatgcggggagtatagttatatgcccggaaaagttcaagacttctttctgtgctcgctccttctgcgcattgtaagtgcaggatggtgtgactgataggcatatatcaccggaagaacttattgcgcttcatgatgcgaatataagccgctacggcggcctgccgggaatgtctgatccgggtagggcagaggccattatcgggagagttcaggccagagttgcctacgaagagatcaccgaccttttcgaagtctccgccacctacctggtggctacagcgagagggcatatattcaatgatgccaataagcgtaccgcgctaaacagtgcgctgctatttctacgccgtaacggggtgcaggtatttgattcacctgaactggcagaccttactgtaggagctgcgactggcgagatatctgtatcttctgtcgccgacacgttacgtagattgtatggttctgcggagtag

SEQ ID NO: 19 - DNA, 1816 bp, synthetic construct
  source 1..1816: mol_type = other DNA
gcccgtcacgggcttctcagggcgttttatggcgggtctgctatgtggtgttatctgactttttgctgttcagcagttcctgccctctgattttccagtctgaccacttcggattatcccgtgacaggtcattcagactggctaatgcacccagtaaggcagcggtatcatcaacaggcttacccgtcttactgtctagactcgaggaattgatatcacccgacaccatcgaatggttatcggttaaccagttccttgttggtggagtccagggtgtcaaacagggatgcaaattcagcatccagcgccgcttttttgtaggcttcgaaagtagccttgctgacaattactgctggctcacggcctctgcgggtgatttcaacctcttccccggcttcaacattgttgagcacttcagaaaggttgccgcgcgcggtacggaagttaatggattgcatagtgaattcctcctgctagcccaaaaaaacgggtatggagaaacagtagagagttgcgataaaaagcgtcaggtaggatccgctaatcttatggataaaaatgctatggcatagcaaagtgtgacgccgtgcaaataatcaatgtggacttttctgccgtgattatagacacttttgttacgcgtttttgtcatggctttggtcccgctttgttacagaatgcttttaataagcggggttaccggtttggttagcgagaagagccagtaaaagacgcagtgacggcaatgtctgatgcaatatggacaattggtttcttctctgaatggcgggagtatgaaaagtatggctgaagcgcaaaatgatcccctgctgccgggatactcgtttaatgcccatctggtggcgggtttaacgccgattgaggccaacggttatctcgatttttttatcgaccgaccgctgggaatgaaaggttatattctcaatctcaccattcgcggtcagggggtggtgaaaaatcagggacgagaatttgtttgccgaccgggtgatattttgctgttcccgccaggagagattcatcactacggtcgtcatccggaggctcgcgaatggtatcaccagtgggtttactttcgtccgcgcgcctactggcatgaatggcttaactggccgtcaatatttgccaatacggggttctttcgcccggatgaagcgcaccagccgcatttcagcgacctgtttgggcaaatcattaacgccgggcaaggggaagggcgctattcggagctgctggcgataaatctgcttgagcaattgttactgcggcgcatggaagcgattaacgagtcgctccatccaccgatggataatcgggtacgcgaggcttgtcagtacatcagcgatcacctggcagacagcaattttgatatcgccagcgtcgcacagcatgtttgcttgtcgccgtcgcgtctgtcacatcttttccgccagcagttagggattagcgtcttaagctggcgcgaggaccaacgtatcagccaggcgaagctgcttttgagcaccacccggatgcctatcgccaccgtcggtcgcaatgttggttttgacgatcaactctatttctcgcgggtatttaaaaaatgcaccggggccagcccgagcgagttccgtgccggttgtgaagaaaaagtgaatgatgtagccgtcaagttgtcataattggtaacgaatcagacaattgacggcttgacggagtagcatagggtttgcagaatccctgcttcgtccatttgacaggcacattatgcatcttggagtggtgaatccgttagcgaggtgccgccggcttccat